European Patent Application EP 4 647 085 A1, published November 12, 2025. Title: FGFR3 발현 또는 활성 억제제의 퇴행성 신경질환 치료 용도. Applicant: 서울대학교 산학협력단. The sequence listing filed with the application follows.

SEQUENCE LISTING (6 sequences)

SEQ ID NO: 1 - protein, 393 aa, synthetic construct
MVVPACVLVFCVAVVAGATSEPPGPEQRVVRRAAEVPGPEPSQQEQVAFGSGDTVELSCHPPGGAPTGPTVWAKDGTGLVASHRILVGPQRLQVLNASHEDAGVYSCQHRLTRRVLCHFSVRVTDAPSSGDDEDGEDVAEDTGAPYWTRPERMDKKLLAVPAANTVRFRCPAAGNPTPSISWLKNGKEFRGEHRIGGIKLRHQQWSLVMESVVPSDRGNYTCVVENKFGSIRQTYTLDVLERSPHRPILQAGLPANQTAILGSDVEFHCKVYSDAQPHIQWLKHVEVNGSKVGPDGTPYVTVLKSWISENVEADARLRLANVSERDGGEYLCRATNFIGVAEKAFWLRVHGPQAAEEELMETDEAGSVYAGVLSYGVVFFLFILVVAAVILCR

SEQ ID NO: 2 - DNA, 29 bp, synthetic construct
  source 1..29: mol_type = other DNA
ccggcctgcgtgctagtgttctgcgtggc

SEQ ID NO: 3 - DNA, 29 bp, synthetic construct
  source 1..29: mol_type = other DNA
tcagtgtgcgtgtaacagatgctccatcc

SEQ ID NO: 4 - DNA, 29 bp, synthetic construct
  source 1..29: mol_type = other DNA
ccggagcgaatggataagaaactgctggc

SEQ ID NO: 5 - DNA, 29 bp, synthetic construct
  source 1..29: mol_type = other DNA
gctgaggaggagctgatggaaactgatga

SEQ ID NO: 6 - DNA, 1989 bp, synthetic construct
  source 1..1989: mol_type = other DNA
atggggagtagcaagagcaagcctaaggaccccagccagcgcctcgacctgcgcagtcccccaaagaagggcttgggctcgcccaccgtgcacaaggtctctcgcttcccgcttaagcgacaggtgtccttggaatctaactcctctatgaactccaacacaccccttgtccggattgcccggctgtcctcaggagaaggtcctgttctggccaatgtttctgaacttgagctgcctgctgaccccaagtgggagctatccaggacccggctgacacttggtaagcctcttggagaaggctgctttggacaggtggtcatggcagaagctattggcatcgacaaggaccgtactgccaagcctgtcaccgtggccgtgaagatgctgaaagatgatgcgactgacaaggacctgtcggacctggtatctgagatggagatgatgaaaatgattggcaagcacaagaacatcattaacctgctgggggcgtgcacacagggtgggcccctgtatgtgctggtggagtacgcagccaagggcaatctccgggagttccttcgggcgcggcggcctccaggcatggactactcctttgatgcctgcaggctgccagaggaacagctcacctgcaaggatctagtgtcctgtgcctaccaggtggcacggggcatggaatacttggcttctcagaagtgtattcacagagacttggctgccagaaacgtcctggtgaccgaggacaatgtgatgaagattgcggactttggcctggctcgagatgtgcacaacctggactactacaagaagaccacaaatggccggctacctgtgaagtggatggcaccagaggccctttttgaccgagtctacacccaccagagtgatgtttggtcttttggtgtcctcctctgggagatctttacgctggggggctcaccgtatcctggcatcccagtggaagagcttttcaagctgttgaaagagggccaccgcatggacaagccagccagctgcacacatgacctgtacatgatcatgcgggaatgttggcatgcggtgccttcacagaggcccaccttcaagcagttggtagaggatttagaccgcatcctcactgtgacatcaaccgacgagtacttggacctctccgtgccgtttgagcagtactcgccaggtggccaggacacgcctagctccagctcgtccggagatgactcggtgttcacccatgacctgctacccccaggtccacccagtaacgggggacctcggacggtcgagggcgtgcaggtggaaaccatctccccaggagacgggcgcaccttccccaagcgcggccagacctgcgtggtgcactacaccgggatgcttgaagatggaaagaaagttgattcctcccgggacagaaacaagccctttaagtttatgctaggcaagcaggaggtgatccgaggctgggaagaaggggttgcccagatgagtgtgggtcagagagccaaactgactatatctccagattatgcctatggtgccactgggcacccaggcatcatcccaccacatgccactctcgtcttcgatgtggagcttctaaaactggaagtcgagggagtgcaggtggaaaccatctccccaggagacgggcgcaccttccccaagcgcggccagacctgcgtggtgcactacaccgggatgcttgaagatggaaagaaagttgattcctcccgggacagaaacaagccctttaagtttatgctaggcaagcaggaggtgatccgaggctgggaagaaggggttgcccagatgagtgtgggtcagagagccaaactgactatatctccagattatgcctatggtgccactgggcacccaggcatcatcccaccacatgccactctcgtcttcgatgtggagcttctaaaactggaatctggcggtggatccggagtcgactatccgtacgacgtaccagactacgcactcgactaa